European Patent Specification EP 3 428 260 B1, published March 13, 2024. Title: VARIANTS AND COMPOSITIONS COMPRISING VARIANTS WITH HIGH STABILITY IN PRESENCE OF A CHELATING AGENT. Applicant: The Procter and Gamble Company. The sequence listing filed with the application follows.

SEQUENCE LISTING (26 sequences)

SEQ ID NO: 1 - DNA, 1440 bp, Bacillus sp.
  CDS (1)..(1440)
gatggattgaacggtacgatgatgcagtattatgagtggcatttggaaaacgacgggcagcattggaatcggttgcacgatgatgccgcagctttgagtgatgctggtattacagctatttggattccgccagcctacaaaggtaatagtcaggcggatgttgggtacggtgcatacgatctttatgatttaggagagttcaatcaaaagggtactgttcgaacgaaatacggaactaaggcacagcttgaacgagctattgggtcccttaaatctaatgatatcaatgtatacggagatgtcgtgatgaatcataaaatgggagctgattttacggaggcagtgcaagctgttcaagtaaatccaacgaatcgttggcaggatatttcaggtgcctacacgattgatgcgtggacgggtttcgacttttcagggcgtaacaacgcctattcagattttaagtggagatggttccattttaatggtgttgactgggatcagcgctatcaagaaaatcatattttccgctttgcaaatacgaactggaactggcgagtggatgaagagaacggtaattatgattacctgttaggatcgaatatcgactttagtcatccagaagtacaagatgagttgaaggattggggtagctggtttaccgatgagttagatttggatggttatcgtttagatgctattaaacatattccattctggtatacatctgattgggttcggcatcagcgcaacgaagcagatcaagatttatttgtcgtaggggaatattggaaggatgacgtaggtgctctcgaattttatttagatgaaatgaattgggagatgtctctattcgatgttccacttaattataatttttaccgggcttcacaacaaggtggaagctatgatatgcgtaatattttacgaggatctttagtagaagcgcatccgatgcatgcagttacgtttgttgataatcatgatactcagccaggggagtcattagagtcatgggttgctgattggtttaagccacttgcttatgcgacaattttgacgcgtgaaggtggttatccaaatgtattttacggtgattactatgggattcctaacgataacatttcagctaaaaaagatatgattgatgagctgcttgatgcacgtcaaaattacgcatatggcacgcagcatgactattttgatcattgggatgttgtaggatggactagggaaggatcttcctccagacctaattcaggccttgcgactattatgtcgaatggacctggtggttccaagtggatgtatgtaggacgtcagaatgcaggacaaacatggacagatttaactggtaataacggagcgtccgttacaattaatggcgatggatggggcgaattctttacgaatggaggatctgtatccgtgtacgtgaaccaa

SEQ ID NO: 2 - protein, 480 aa, Bacillus sp.
DGLNGTMMQYYEWHLENDGQHWNRLHDDAAALSDAGITAIWIPPAYKGNSQADVGYGAYDLYDLGEFNQKGTVRTKYGTKAQLERAIGSLKSNDINVYGDVVMNHKMGADFTEAVQAVQVNPTNRWQDISGAYTIDAWTGFDFSGRNNAYSDFKWRWFHFNGVDWDQRYQENHIFRFANTNWNWRVDEENGNYDYLLGSNIDFSHPEVQDELKDWGSWFTDELDLDGYRLDAIKHIPFWYTSDWVRHQRNEADQDLFVVGEYWKDDVGALEFYLDEMNWEMSLFDVPLNYNFYRASQQGGSYDMRNILRGSLVEAHPMHAVTFVDNHDTQPGESLESWVADWFKPLAYATILTREGGYPNVFYGDYYGIPNDNISAKKDMIDELLDARQNYAYGTQHDYFDHWDVVGWTREGSSSRPNSGLATIMSNGPGGSKWMYVGRQNAGQTWTDLTGNNGASVTINGDGWGEFFTNGGSVSVYVNQ

SEQ ID NO: 3 - DNA, 1476 bp, Bacillus circulans
  CDS (1)..(1476)
aagagaaatcataccatgatgcagttttttgaatggcacctggctgcagacggagatcattggaagcgactggctgaaatggccccggaattgaaagccaaaggcattgatacggtatgggtgcctcctgtgaccaaagccgtatcagctgaggatacaggttatggtgtatatgatctgtatgatttgggtgaatttgaccaaaagggtaccgtgcgtaccaaatacggcaccaagcaggaactgatagaggccattgctgagtgtcagaagaacggaatcgccgtctatgtggatctggttatgaatcacaaggccggagcagatgagacggaagtttttaaagtgattgaggttgatcccaatgatcgaacgaaggaaatttctgagccgttcgaaattgagggctggaccaaattcacattcccgggtcgcggggatcaatactcctcttttaaatggaactctgaacacttcaatggcacggactttgatgccagggaagaacgaacaggtgtattccgcatcgcaggagagaataaaaaatggaatgagaatgtcgatgatgagtttggtaactatgactatctgatgttcgccaatatagattataaccacccggatgttcggcgcgagatgatcgattgggggaaatggctgatcgatacccttcagtgcggtgggttccggctggatgcgattaagcatatcaaccatgaattcattaaggagttcgcagcagagatgatccgcaaacgcggtcaggatttctacatcgtaggcgagttctggaactcgaacctggatgcatgtcgtgaattccttgatacggtagactatcagatcgacctgtttgatgtgtctcttcactacaagttgcatgaggcttcgcttaaaggcagagactttgatctctccaaaatttttgatgacaccttggtgcagacccatcctacccatgcggtaaccttcgtagataaccatgactcccaacctcatgaagcgttggaatcatggattggtgattggtttaagccgagcgcttatgcgttgacgctattacgtcgtgatggctatccggttgtattttacggcgattattatggcattggtggtcctgaacctgtggatggcaaaaaagaaattctggacattctgctgtctgcccgttgcaacaaagcgtatggagagcaggaagattacttcgatcacgccaatacgattggctgggtacgtcgtggcgtagaggaaatcgaaggttccggttgtgcagtggtcatctccaacggggatgacggtgagaagagaatgttcatcggagagcatcgtgctggtgaagtctgggtggatctgacgaagagctgtgatgatcagattaccattgaggaagacggctgggccaccttccatgtgtgcggtggaggtgtctcggtatgggctcttcctgaacagaatgaggactgcgctgacgctgag

SEQ ID NO: 4 - protein, 492 aa, Bacillus circulans
KRNHTMMQFFEWHLAADGDHWKRLAEMAPELKAKGIDTVWVPPVTKAVSAEDTGYGVYDLYDLGEFDQKGTVRTKYGTKQELIEAIAECQKNGIAVYVDLVMNHKAGADETEVFKVIEVDPNDRTKEISEPFEIEGWTKFTFPGRGDQYSSFKWNSEHFNGTDFDAREERTGVFRIAGENKKWNENVDDEFGNYDYLMFANIDYNHPDVRREMIDWGKWLIDTLQCGGFRLDAIKHINHEFIKEFAAEMIRKRGQDFYIVGEFWNSNLDACREFLDTVDYQIDLFDVSLHYKLHEASLKGRDFDLSKIFDDTLVQTHPTHAVTFVDNHDSQPHEALESWIGDWFKPSAYALTLLRRDGYPVVFYGDYYGIGGPEPVDGKKEILDILLSARCNKAYGEQEDYFDHANTIGWVRRGVEEIEGSGCAVVISNGDDGEKRMFIGEHRAGEVWVDLTKSCDDQITIEEDGWATFHVCGGGVSVWALPEQNEDCADAE

SEQ ID NO: 5 - DNA, 1455 bp, bacillus sp.
  CDS (1)..(1455)
catcataatgggacaaatgggacgatgatgcaatactttgaatggcacttgcctaatgatgggaatcactggaatagattaagagatgatgctagtaatctaagaaatagaggtataaccgctatttggattccgcctgcctggaaagggacttcgcaaaatgatgtggggtatggagcctatgatctttacgatttaggggaatttaatcaaaaggggacggttcgtactaagtatgggacacgtagtcaattggagtctgccatccatgctttaaagaataatggcgttcaagtttatggggatgtagtgatgaaccataaaggaggagctgatgctacagaaaacgttcttgctgtcgaggtgaatccaaataaccggaatcaagaaatatctggggactacacaattgaggcttggactaagtttgattttccagggaggggtaatacatactcagactttaaatggcgttggtatcatttcgatggtgtagattgggatcaatcacgacaattccaaaatcgtatctacaaattccgaggtgatggcaaagcttgggattgggaagtagattcggaaaatggaaattatgattatttaatgtatgcagatgtagatatggatcatccggaggtagtaaatgagcttagaagatggggagaatggtatacaaatacattaaatcttgatggatttaggatcgatgcggtgaagcatattaaatatagctttacacgtgattggttgacccatgtaagaaacgcaacgggaaaagaaatgtttgctgttgctgaattttggaaaaatgatttaggtgccttggagaactatttaaataaaacaaactggaatcattctgtctttgatgtcccccttcattataatctttataacgcgtcaaatagtggaggcaactatgacatggcaaaacttcttaatggaacggttgttcaaaagcatccaatgcatgccgtaacttttgtggataatcacgattctcaacctggggaatcattagaatcatttgtacaagaatggtttaagccacttgcttatgcgcttattttaacaagagaacaaggctatccctctgtcttctatggtgactactatggaattccaacacatagtgtcccagcaatgaaagccaagattgatccaatcttagaggcgcgtcaaaattttgcatatggaacacaacatgattattttgaccatcataatataatcggatggacacgtgaaggaaataccacgcatcccaattcaggacttgcgactatcatgtcggatgggccagggggagagaaatggatgtacgtagggcaaaataaagcaggtcaagtttggcatgacataactggaaataaaccaggaacagttacgatcaatgcagatggatgggctaatttttcagtaaatggaggatctgtttccatttgggtgaaacga

SEQ ID NO: 6 - protein, 485 aa, bacillus sp.
HHNGTNGTMMQYFEWHLPNDGNHWNRLRDDASNLRNRGITAIWIPPAWKGTSQNDVGYGAYDLYDLGEFNQKGTVRTKYGTRSQLESAIHALKNNGVQVYGDVVMNHKGGADATENVLAVEVNPNNRNQEISGDYTIEAWTKFDFPGRGNTYSDFKWRWYHFDGVDWDQSRQFQNRIYKFRGDGKAWDWEVDSENGNYDYLMYADVDMDHPEVVNELRRWGEWYTNTLNLDGFRIDAVKHIKYSFTRDWLTHVRNATGKEMFAVAEFWKNDLGALENYLNKTNWNHSVFDVPLHYNLYNASNSGGNYDMAKLLNGTVVQKHPMHAVTFVDNHDSQPGESLESFVQEWFKPLAYALILTREQGYPSVFYGDYYGIPTHSVPAMKAKIDPILEARQNFAYGTQHDYFDHHNIIGWTREGNTTHPNSGLATIMSDGPGGEKWMYVGQNKAGQVWHDITGNKPGTVTINADGWANFSVNGGSVSIWVKR

SEQ ID NO: 7 - DNA, 1455 bp, Bacillus sp.
  CDS (1)..(1455)
catcataacggtacgaacgggacaatgatgcaatactttgaatggtatctacctaatgacggaaatcattggaatcgattaaactctgatgcgagtaaccttaaaagcaaagggattacagcggtgtggattcctccagcatggaagggcgcttctcaaaatgacgtaggatacggagcctatgacctgtatgatctgggagaatttaatcaaaaaggtaccgtccgtacaaaatatggaacacgtagtcagttacaagctgcggtaacctccttaaaaaataatggaattcaagtatatggtgacgttgttatgaatcacaaaggtggcgcagacgctactgaaatggtaagggccgttgaagtgaatcccaataaccgtaaccaagaagtgactggtgaatataccattgaagcttggactagatttgattttccagggcgaggaaatactcattctagctttaaatggagatggtatcattttgatggtgtggattgggatcagtcacgtagactgaacaatcgcatctataaatttagaggtcatggcaaagcttgggattgggaagttgatacggaaaatggtaattatgattatttaatgtacgctgatattgatatggatcacccagaagtagtaaatgaattaagaaattggggtgtttggtacacaaacacattaggactcgatggatttagaatagatgcggttaaacatataaagtatagctttacgcgcgattggattaatcacgttagaagtgcaacaggtaaaaatatgtttgcggttgctgagttttggaagaatgatttaggtgcaattgaaaactatctgcagaaaacaaactggaaccattcagtctttgatgtgccgttacattataatctttataatgcatcaaaaagcggagggaactatgatatgcgaaacatatttaatggaacggttgttcaacgacatccaagtcatgctgtaacatttgttgataatcatgattcgcagcctgaagaagcattagaatcttttgttgaagaatggtttaaaccattagcgtatgcgcttacattaacgcgtgaacaaggatacccttctgtattttacggagattattatgggattccaacacatggagtgccagcaatgagatcaaaaatcgatccgattttagaagcacgtcaaaagtatgcatacggaaaacaaaatgattacttagaccatcataatatcattggttggacgcgtgaagggaatacagcacaccccaattcaggtctagctaccatcatgtctgatggagcgggtggaagtaagtggatgtttgttgggcgtaataaggctggtcaagtatggagtgatattacaggaaaccgtacaggtacggttacaatcaatgcagacggttggggcaatttctctgtgaatggagggtcagtttctatttgggtcaacaaa

SEQ ID NO: 8 - protein, 485 aa, Bacillus sp.
HHNGTNGTMMQYFEWYLPNDGNHWNRLNSDASNLKSKGITAVWIPPAWKGASQNDVGYGAYDLYDLGEFNQKGTVRTKYGTRSQLQAAVTSLKNNGIQVYGDVVMNHKGGADATEMVRAVEVNPNNRNQEVTGEYTIEAWTRFDFPGRGNTHSSFKWRWYHFDGVDWDQSRRLNNRIYKFRGHGKAWDWEVDTENGNYDYLMYADIDMDHPEVVNELRNWGVWYTNTLGLDGFRIDAVKHIKYSFTRDWINHVRSATGKNMFAVAEFWKNDLGAIENYLQKTNWNHSVFDVPLHYNLYNASKSGGNYDMRNIFNGTVVQRHPSHAVTFVDNHDSQPEEALESFVEEWFKPLAYALTLTREQGYPSVFYGDYYGIPTHGVPAMRSKIDPILEARQKYAYGKQNDYLDHHNIIGWTREGNTAHPNSGLATIMSDGAGGSKWMFVGRNKAGQVWSDITGNRTGTVTINADGWGNFSVNGGSVSIWVNK

SEQ ID NO: 9 - DNA, 1458 bp, Bacillus sp.
  CDS (1)..(1458)
caccataatggtacgaacggcacaatgatgcagtactttgaatggtatctaccaaatgacggaaaccattggaatagattaaggtctgatgcaagtaacctaaaagataaagggatctcagcggtttggattcctcctgcatggaagggtgcctctcaaaatgatgtggggtatggtgcttatgatctgtatgatttaggagaattcaatcaaaaaggaaccattcgtacaaaatatggaacgcgcaatcagttacaagctgcagttaacgccttgaaaagtaatggaattcaagtgtatggcgatgttgtaatgaatcataaagggggagcagacgctaccgaaatggttagggcggttgaagtaaacccgaataatagaaatcaagaagtgtccggtgaatatacaattgaggcttggacaaagtttgactttcctggacgaggtaatacccattcaaacttcaaatggagatggtatcactttgatggagtagattgggatcagtcacgtaagctgaacaatcgaatttataaatttagaggtgatggaaaagggtgggattgggaagtcgatacagaaaacggtaactatgattacctaatgtatgcagatattgacatggatcacccagaggtagtgaatgagctaagaaattggggtgtttggtatacgaatacattaggccttgatggttttagaatagatgcagtaaaacatataaaatacagctttactcgtgattggatcaatcatgttagaagtgcaactggcaaaaatatgtttgcggttgcggaattttggaaaaatgatttaggtgctattgaaaactatttaaacaaaacaaactggaaccattcagtctttgatgttccgctgcactataacctctataatgcttcaaaaagcggagggaattatgatatgaggcaaatatttaatggtacagtcgtgcaaagacatccaatgcatgctgttacatttgttgataatcatgattcgcaacctgaagaagctttagagtcttttgttgaagaatggttcaaaccattagcgtatgctttgacattaacacgtgaacaaggctacccttctgtattttatggagattattatggcattccaacgcatggtgtaccagcgatgaaatcgaaaattgacccgattctagaagcgcgtcaaaagtatgcatatggaagacaaaatgactacttagaccatcataatatcattggttggacacgtgaagggaatacagcacaccccaactctggtttagctactatcatgtccgatggagcaggaggaaataagtggatgtttgttgggcgtaataaagctggtcaagtttggaccgatatcactggaaatcgtgcaggtactgttacgattaatgctgatggatggggtaatttttctgtaaatggaggatcagtttctatttgggtaaacaaataa

SEQ ID NO: 10 - protein, 485 aa, Bacillus sp.
HHNGTNGTMMQYFEWYLPNDGNHWNRLRSDASNLKDKGISAVWIPPAWKGASQNDVGYGAYDLYDLGEFNQKGTIRTKYGTRNQLQAAVNALKSNGIQVYGDVVMNHKGGADATEMVRAVEVNPNNRNQEVSGEYTIEAWTKFDFPGRGNTHSNFKWRWYHFDGVDWDQSRKLNNRIYKFRGDGKGWDWEVDTENGNYDYLMYADIDMDHPEVVNELRNWGVWYTNTLGLDGFRIDAVKHIKYSFTRDWINHVRSATGKNMFAVAEFWKNDLGAIENYLNKTNWNHSVFDVPLHYNLYNASKSGGNYDMRQIFNGTVVQRHPMHAVTFVDNHDSQPEEALESFVEEWFKPLAYALTLTREQGYPSVFYGDYYGIPTHGVPAMKSKIDPILEARQKYAYGRQNDYLDHHNIIGWTREGNTAHPNSGLATIMSDGAGGNKWMFVGRNKAGQVWTDITGNRAGTVTINADGWGNFSVNGGSVSIWVNK

SEQ ID NO: 11 - DNA, 1455 bp, Bacillus Sp
  CDS (1)..(1455)
catcataatggaacaaatggtactatgatgcaatatttcgaatggtatttgccaaatgacgggaatcattggaacaggttgagggatgacgcagctaacttaaagagtaaagggataacagctgtatggattccacctgcatggaaggggacttcccagaatgatgtaggttatggagcctatgatttatatgatcttggagagtttaaccagaaggggacggttcgtacaaaatatggaacacgcaaccagctgcaggctgccgtgacatctttaaaaaataacggcattcaggtatatggtgatgtcgtcatgaatcataaaggtggagcagatggtacggaaattgtaaatgcggtagaagtgaatcggagcaaccgaaaccaggaaacctcaggagagtatgcaatagaagcgtggacaaagtttgattttcctggaagaggaaataaccattccagctttaagtggcgctggtatcattttgatgggacagattgggatcagtcacgccagcttcaaaacaaaatatataaattcaggggaacaggcaaggcctgggactgggaagtcgatacagagaatggcaactatgactatcttatgtatgcagacgtggatatggatcacccagaagtaatacatgaacttagaaactggggagtgtggtatacgaatacactgaaccttgatggatttagaatagatgcagtgaaacatataaaatatagctttacgagagattggcttacacatgtgcgtaacaccacaggtaaaccaatgtttgcagtggctgagttttggaaaaatgaccttggtgcaattgaaaactatttgaataaaacaagttggaatcactcggtgtttgatgttcctctccactataatttgtacaatgcatctaatagcggtggttattatgatatgagaaatattttaaatggttctgtggtgcaaaaacatccaacacatgccgttacttttgttgataaccatgattctcagcccggggaagcattggaatcctttgttcaacaatggtttaaaccacttgcatatgcattggttctgacaagggaacaaggttatccttccgtattttatggggattactacggtatcccaacccatggtgttccggctatgaaatctaaaatagaccctcttctgcaggcacgtcaaacttttgcctatggtacgcagcatgattactttgatcatcatgatattatcggttggacaagagagggaaatagctcccatccaaattcaggccttgccaccattatgtcagatggtccaggtggtaacaaatggatgtatgtggggaaaaataaagcgggacaagtttggagagatattaccggaaataggacaggcaccgtcacaattaatgcagacggatggggtaatttctctgttaatggagggtccgtttcggtttgggtgaagcaa

SEQ ID NO: 12 - protein, 485 aa, Bacillus Sp
HHNGTNGTMMQYFEWYLPNDGNHWNRLRDDAANLKSKGITAVWIPPAWKGTSQNDVGYGAYDLYDLGEFNQKGTVRTKYGTRNQLQAAVTSLKNNGIQVYGDVVMNHKGGADGTEIVNAVEVNRSNRNQETSGEYAIEAWTKFDFPGRGNNHSSFKWRWYHFDGTDWDQSRQLQNKIYKFRGTGKAWDWEVDTENGNYDYLMYADVDMDHPEVIHELRNWGVWYTNTLNLDGFRIDAVKHIKYSFTRDWLTHVRNTTGKPMFAVAEFWKNDLGAIENYLNKTSWNHSVFDVPLHYNLYNASNSGGYYDMRNILNGSVVQKHPTHAVTFVDNHDSQPGEALESFVQQWFKPLAYALVLTREQGYPSVFYGDYYGIPTHGVPAMKSKIDPLLQARQTFAYGTQHDYFDHHDIIGWTREGNSSHPNSGLATIMSDGPGGNKWMYVGKNKAGQVWRDITGNRTGTVTINADGWGNFSVNGGSVSVWVKQ

SEQ ID NO: 13 - DNA, 1452 bp, Bacillus amyloliquefaciens
  CDS (1)..(1449)
gtaaatggcacgctgatgcagtattttgaatggtatacgccgaacgacggccagcattggaaacgattgcagaatgatgcggaacatttatcggatatcggaatcactgccgtctggattcctcccgcatacaaaggattgagccaatccgataacggatacggaccttatgatttgtatgatttaggagaattccagcaaaaagggacggtcagaacgaaatacggcacaaaatcagagcttcaagatgcgatcggctcactgcattcccggaacgtccaagtatacggagatgtggttttgaatcataaggctggtgctgatgcaacagaagatgtaactgccgtcgaagtcaatccggccaatagaaatcaggaaacttcggaggaatatcaaatcaaagcgtggacggattttcgttttccgggccgtggaaacacgtacagtgattttaaatggcattggtatcatttcgacggagcggactgggatgaatcccggaagatcagccgcatctttaagtttcgtggggaaggaaaagcgtgggattgggaagtatcaagtgaaaacggcaactatgactatttaatgtatgctgatgttgactacgaccaccctgatgtcgtggcagagacaaaaaaatggggtatctggtatgcgaatgaactgtcattagacggcttccgtattgatgccgccaaacatattaaattttcatttctgcgtgattgggttcaggcggtcagacaggcgacgggaaaagaaatgtttacggttgcggagtattggcagaataatgccgggaaactcgaaaactacttgaataaaacaagctttaatcaatccgtgtttgatgttccgcttcatttcaatttacaggcggcttcctcacaaggaggcggatatgatatgaggcgtttgctggacggtaccgttgtgtccaggcatccggaaaaggcggttacatttgttgaaaatcatgacacacagccgggacagtcattggaatcgacagtccaaacttggtttaaaccgcttgcatacgcctttattttgacaagagaatccggttatcctcaggtgttctatggggatatgtacgggacaaaagggacatcgccaaaggaaattccctcactgaaagataatatagagccgattttaaaagcgcgtaaggagtacgcatacgggccccagcacgattatattgaccacccggatgtgatcggatggacgagggaaggtgacagctccgccgccaaatcaggtttggccgctttaatcacggacggacccggcggatcaaagcggatgtatgccggcctgaaaaatgccggcgagacatggtatgacataacgggcaaccgttcagatactgtaaaaatcggatctgacggctggggagagtttcatgtaaacgatgggtccgtctccatttatgttcagaaataa

SEQ ID NO: 14 - protein, 483 aa, Bacillus amyloliquefaciens
VNGTLMQYFEWYTPNDGQHWKRLQNDAEHLSDIGITAVWIPPAYKGLSQSDNGYGPYDLYDLGEFQQKGTVRTKYGTKSELQDAIGSLHSRNVQVYGDVVLNHKAGADATEDVTAVEVNPANRNQETSEEYQIKAWTDFRFPGRGNTYSDFKWHWYHFDGADWDESRKISRIFKFRGEGKAWDWEVSSENGNYDYLMYADVDYDHPDVVAETKKWGIWYANELSLDGFRIDAAKHIKFSFLRDWVQAVRQATGKEMFTVAEYWQNNAGKLENYLNKTSFNQSVFDVPLHFNLQAASSQGGGYDMRRLLDGTVVSRHPEKAVTFVENHDTQPGQSLESTVQTWFKPLAYAFILTRESGYPQVFYGDMYGTKGTSPKEIPSLKDNIEPILKARKEYAYGPQHDYIDHPDVIGWTREGDSSAAKSGLAALITDGPGGSKRMYAGLKNAGETWYDITGNRSDTVKIGSDGWGEFHVNDGSVSIYVQK

SEQ ID NO: 15 - DNA, 1548 bp, Bacillus stearothermophilus
  CDS (1)..(1548)
gccgcaccgtttaacggcaccatgatgcagtattttgaatggtacttgccggatgatggcacgttatggaccaaagtggccaatgaagccaacaacttatccagccttggcatcaccgctctttggctgccgcccgcttacaaaggaacaagccgcagcgacgtagggtacggagtatacgacttgtatgacctcggcgaattcaatcaaaaagggaccgtccgcacaaaatacggaacaaaagctcaatatcttcaagccattcaagccgcccacgccgctggaatgcaagtgtacgccgatgtcgtgttcgaccataaaggcggcgctgacggcacggaatgggtggacgccgtcgaagtcaatccgtccgaccgcaaccaagaaatctcgggcacctatcaaatccaagcatggacgaaatttgattttcccgggcggggcaacacctactccagctttaagtggcgctggtaccattttgacggcgttgattgggacgaaagccgaaaattgagccgcatttacaaattccgcggcatcggcaaagcgtgggattgggaagtagacacggaaaacggaaactatgactacttaatgtatgccgaccttgatatggatcatcccgaagtcgtgaccgagctgaaaaactgggggaaatggtatgtcaacacaacgaacattgatgggttccggcttgatgccgtcaagcatattaagttcagtttttttcctgattggttgtcgtatgtgcgttctcagactggcaagccgctatttaccgtcggggaatattggagctatgacatcaacaagttgcacaattacattacgaaaacagacggaacgatgtctttgtttgatgccccgttacacaacaaattttataccgcttccaaatcagggggcgcatttgatatgcgcacgttaatgaccaatactctcatgaaagatcaaccgacattggccgtcaccttcgttgataatcatgacaccgaacccggccaagcgctgcagtcatgggtcgacccatggttcaaaccgttggcttacgcctttattctaactcggcaggaaggatacccgtgcgtcttttatggtgactattatggcattccacaatataacattccttcgctgaaaagcaaaatcgatccgctcctcatcgcgcgcagggattatgcttacggaacgcaacatgattatcttgatcactccgacatcatcgggtggacaagggaagggggcactgaaaaaccaggatccggactggccgcactgatcaccgatgggccgggaggaagcaaatggatgtacgttggcaaacaacacgctggaaaagtgttctatgaccttaccggcaaccggagtgacaccgtcaccatcaacagtgatggatggggggaattcaaagtcaatggcggttcggtttcggtttgggttcctagaaaaacgaccgtttctaccatcgctcggccgatcacaacccgaccgtggactggtgaattcgtccgttggaccgaaccacggttggtggcatggccttga

SEQ ID NO: 16 - protein, 515 aa, Bacillus stearothermophilus
AAPFNGTMMQYFEWYLPDDGTLWTKVANEANNLSSLGITALWLPPAYKGTSRSDVGYGVYDLYDLGEFNQKGTVRTKYGTKAQYLQAIQAAHAAGMQVYADVVFDHKGGADGTEWVDAVEVNPSDRNQEISGTYQIQAWTKFDFPGRGNTYSSFKWRWYHFDGVDWDESRKLSRIYKFRGIGKAWDWEVDTENGNYDYLMYADLDMDHPEVVTELKNWGKWYVNTTNIDGFRLDAVKHIKFSFFPDWLSYVRSQTGKPLFTVGEYWSYDINKLHNYITKTDGTMSLFDAPLHNKFYTASKSGGAFDMRTLMTNTLMKDQPTLAVTFVDNHDTEPGQALQSWVDPWFKPLAYAFILTRQEGYPCVFYGDYYGIPQYNIPSLKSKIDPLLIARRDYAYGTQHDYLDHSDIIGWTREGGTEKPGSGLAALITDGPGGSKWMYVGKQHAGKVFYDLTGNRSDTVTINSDGWGEFKVNGGSVSVWVPRKTTVSTIARPITTRPWTGEFVRWTEPRLVAWP

SEQ ID NO: 17 - DNA, 1455 bp, bacillus sp.
  CDS (1)..(1455)
catcataatgggacgaatgggaccatgatgcagtattttgaatggcatttgccaaatgacgggaaccactggaacaggttacgagatgacgcagctaacttaaagagtaaagggattaccgctgtttggattcctcctgcatggaaggggacttcgcaaaatgatgttgggtatggtgcctatgatttgtacgatcttggtgagtttaaccaaaagggaaccgtccgtacaaaatatggcacaaggagtcagttgcaaggtgccgtgacatctttgaaaaataacgggattcaagtttatggggatgtcgtgatgaatcataaaggtggagcagacgggacagagatggtaaatgcggtggaagtgaaccgaagcaaccgaaaccaagaaatatcaggtgaatacaccattgaagcatggacgaaatttgatttccctggaagaggaaatacccattccaactttaaatggcgctggtatcattttgatgggacagattgggatcagtcacgtcagcttcagaacaaaatatataaattcagaggtaccggaaaggcatgggactgggaagtagatatagagaacggcaactatgattaccttatgtatgcagacattgatatggatcatccagaagtaatcaatgaacttagaaattggggagtttggtatacaaatacacttaatctagatggatttagaatcgatgctgtgaaacatattaaatacagctatacgagagattggctaacacatgtgcgtaacaccacaggtaaaccaatgtttgcagttgcagaattttggaaaaatgaccttgctgcaatcgaaaactatttaaataaaacaagttggaatcactccgtgttcgatgttcctcttcattataatttgtacaatgcatctaatagtggtggctattttgatatgagaaatattttaaatggttctgtcgtacaaaaacaccctatacatgcagtcacatttgttgataaccatgactctcagccaggagaagcattggaatcctttgttcaatcgtggttcaaaccactggcatatgcattgattctgacaagggagcaaggttacccttccgtattttacggtgattactacggtataccaactcatggtgttccttcgatgaaatctaaaattgatccacttctgcaggcacgtcaaacgtatgcctacggaacccaacatgattattttgatcatcatgatattatcggctggacgagagaaggggacagctcccacccaaattcaggacttgcaactattatgtccgatgggccagggggtaataaatggatgtatgtcgggaaacataaagctggccaagtatggagagatatcaccggaaataggtctggtaccgtcaccattaatgcagatggttgggggaatttcactgtaaacggaggggcagtttcggtttgggtgaagcaa

SEQ ID NO: 18 - protein, 485 aa, bacillus sp.
HHNGTNGTMMQYFEWHLPNDGNHWNRLRDDAANLKSKGITAVWIPPAWKGTSQNDVGYGAYDLYDLGEFNQKGTVRTKYGTRSQLQGAVTSLKNNGIQVYGDVVMNHKGGADGTEMVNAVEVNRSNRNQEISGEYTIEAWTKFDFPGRGNTHSNFKWRWYHFDGTDWDQSRQLQNKIYKFRGTGKAWDWEVDIENGNYDYLMYADIDMDHPEVINELRNWGVWYTNTLNLDGFRIDAVKHIKYSYTRDWLTHVRNTTGKPMFAVAEFWKNDLAAIENYLNKTSWNHSVFDVPLHYNLYNASNSGGYFDMRNILNGSVVQKHPIHAVTFVDNHDSQPGEALESFVQSWFKPLAYALILTREQGYPSVFYGDYYGIPTHGVPSMKSKIDPLLQARQTYAYGTQHDYFDHHDIIGWTREGDSSHPNSGLATIMSDGPGGNKWMYVGKHKAGQVWRDITGNRSGTVTINADGWGNFTVNGGAVSVWVKQ

SEQ ID NO: 19 - DNA, 1452 bp, Bacillus licheniformis
  CDS (1)..(1452)
gcaaatcttaatgggacgctgatgcagtattttgaatggtacatgcccaatgacggccaacattggaggcgtttgcaaaacgactcggcatatttggctgaacacggtattactgccgtctggattcccccggcatataagggaacgagccaagcggatgtgggctacggtgcttacgacctttatgatttaggggagtttcatcaaaaagggacggttcggacaaagtacggcacaaaaggagagctgcaatctgcgatcaaaagtcttcattcccgcgacattaacgtttacggggatgtggtcatcaaccacaaaggcggcgctgatgcgaccgaagatgtaaccgcggttgaagtcgatcccgctgaccgcaaccgcgtaatttcaggagaacacctaattaaagcctggacacattttcattttccggggcgcggcagcacatacagcgattttaaatggcattggtaccattttgacggaaccgattgggacgagtcccgaaagctgaaccgcatctataagtttcaaggaaaggcttgggattgggaagtttccaatgaaaacggcaactatgattatttgatgtatgccgacatcgattatgaccatcctgatgtcgcagcagaaattaagagatggggcacttggtatgccaatgaactgcaattggacggtttccgtcttgatgctgtcaaacacattaaattttcttttttgcgggattgggttaatcatgtcagggaaaaaacggggaaggaaatgtttacggtagctgaatattggcagaatgacttgggcgcgctggaaaactatttgaacaaaacaaattttaatcattcagtgtttgacgtgccgcttcattatcagttccatgctgcatcgacacagggaggcggctatgatatgaggaaattgctgaacggtacggtcgtttccaagcatccgttgaaatcggttacatttgtcgataaccatgatacacagccggggcaatcgcttgagtcgactgtccaaacatggtttaagccgcttgcttacgcttttattctcacaagggaatctggataccctcaggttttctacggggatatgtacgggacgaaaggagactcccagcgcgaaattcctgccttgaaacacaaaattgaaccgatcttaaaagcgagaaaacagtatgcgtacggagcacagcatgattatttcgaccaccatgacattgtcggctggacaagggaaggcgacagctcggttgcaaattcaggtttggcggcattaataacagacggacccggtggggcaaagcgaatgtatgtcggccggcaaaacgccggtgagacatggcatgacattaccggaaaccgttcggagccggttgtcatcaattcggaaggctggggagagtttcacgtaaacggcgggtcggtttcaatttatgttcaaagatag

SEQ ID NO: 20 - protein, 483 aa, Bacillus licheniformis [sequence omitted]

SEQ ID NO: 21 - DNA, 1455 bp, bacillus sp.
  CDS (1)..(1455)
caccataatggcacaaatggaacaatgatgcaatattttgaatggtatttgccaaatgacggtaatcattggaatagattaagatcagatgcaagtaatcttaaagataaagggattacagcggtttggattccacctgcttggaaaggggcttctcaaaatgatgtagggtatggagcctatgatctgtatgatttaggagaattcaatcaaaaaggaaccgtacgtacaaagtacggaacccgtaatcaattacaagctgcagtaaccgccttaaaaagtaatggtattcaagtatacggagatgtcgtaatgaatcataagggtggagcggatgccactgagtgggttcgagcggttgaagtgaacccaagtaatcgtaatcaagaagtctctggtgattatacgattgaggcttggactaagtttgattttcctggtcgaggtaatacccactctaactttaaatggagatggtatcatttcgatggtgtagattgggatcagtcacgtcaattgcagaatcgaatctataaattcagaggagatggaaaaggttgggactgggaagttgatacagagaacggaaactatgactatctaatgtacgcggatattgatatggatcaccctgaagtagtgaatgaactcagaaactggggtgtatggtataccaatacactggggctagacgggttcagaatagatgcggtaaaacatataaaatatagctttactcgtgattggcttactcacgttagaaatacgacaggtaaaaatatgtttgcagttgcagagttctggaagaatgacataggtgcaattgaaaattacttaagtaaaacaaattggaatcattcagtttttgatgtgcccctgcattataacctttataatgcatcgagaagtggtggcaattatgatatgaggcaaatatttaatggaacagttgttcagagacatcctacacatgctgtaacatttgttgataaccatgattcacagccggaagaagccctagagtcatttgttgaagagtggttcaaaccgttagcgtatgctctcacactaacacgtgatcaaggatatccttccgttttttatggagattattatgggattccgacgcatggtgtaccagcaatgaaatctaagattgatccgattttagaagcacgtcaaaagtatgcgtacggaaaacaaaatgattatttggatcaccataatatgattggctggacgcgtgaaggtaatacagcacatcccaactcaggactagcaactattatgtcggatggcccaggaggaaataaatggatgtatgttgggcgtaataaggctggacaagtttggagagatattacaggaaatcgctcaggtacggtgacgattaacgcagatgggtggggtaatttttctgtaaatggtgggtctgtatctatatgggtaaataat

SEQ ID NO: 22 - protein, 485 aa, bacillus sp.
HHNGTNGTMMQYFEWYLPNDGNHWNRLRSDASNLKDKGITAVWIPPAWKGASQNDVGYGAYDLYDLGEFNQKGTVRTKYGTRNQLQAAVTALKSNGIQVYGDVVMNHKGGADATEWVRAVEVNPSNRNQEVSGDYTIEAWTKFDFPGRGNTHSNFKWRWYHFDGVDWDQSRQLQNRIYKFRGDGKGWDWEVDTENGNYDYLMYADIDMDHPEVVNELRNWGVWYTNTLGLDGFRIDAVKHIKYSFTRDWLTHVRNTTGKNMFAVAEFWKNDIGAIENYLSKTNWNHSVFDVPLHYNLYNASRSGGNYDMRQIFNGTVVQRHPTHAVTFVDNHDSQPEEALESFVEEWFKPLAYALTLTRDQGYPSVFYGDYYGIPTHGVPAMKSKIDPILEARQKYAYGKQNDYLDHHNMIGWTREGNTAHPNSGLATIMSDGPGGNKWMYVGRNKAGQVWRDITGNRSGTVTINADGWGNFSVNGGSVSIWVNN

SEQ ID NO: 23 - DNA, 1452 bp, bacillus sp
  CDS (1)..(1452)
ggaagtgtgccggtaaatggcacaatgatgcaatatttcgaatggtaccttccagacgatggaacactatggacgaaagtagcaaataacgctcaatctttagcgaatcttggcattactgccctttggcttccccctgcctataaaggaacaagcagcagtgacgttggatatggcgtttatgatttatatgaccttggagagtttaatcaaaaaggaactgtccgaacaaaatacgggacaaaaacacaatatatccaagcaatccaagcggcgcatacagcagggatgcaagtatatgcagatgtcgtctttaaccataaagccggtgcagatggaacagaactagtcgatgcagtagaagtaaatccttctgaccgcaatcaagaaatatcaggaacatatcaaatccaagcgtggacaaaatttgattttcctggtcgtggaaacacctattctagttttaaatggcgttggtatcatttcgatggaacggactgggatgagagtagaaaactaaatcgtatttacaagttccgcggcacgggaaaagcatgggattgggaagtagatacagaaaacgggaattatgactatctcatgtatgcagatttagatatggatcatccagaggttgtatccgaactaaaaaattggggaaagtggtatgtaaccacaaccaatatcgacggattccgtctggatgcagtgaagcatattaaatatagctttttcccggactggctatcgtacgtacgaacccaaacacaaaagcctctttttgccgttggggaattttggagctatgacattagcaagttgcacaactatattacaaagacgaacggctctatgtccctattcgatgccccgctgcataacaatttttatatagcatcgaaatcaggcggttattttgatatgcgcacattactcaacaacacattgatgaaagatcagcctacattagcagtcacattagtggataatcacgatactgagccagggcaatctctgcagtcatgggtcgagccatggtttaaaccgttagcttacgcatttatcttgacccgccaagaaggttatccttgcgtcttttatggagattactatggtattccaaaatacaacattcctgcgctgaaaagcaaacttgatccgctgttaattgccagaagagattatgcctatggaacacagcacgactatattgacagtgcggatattatcggttggacgcgggaaggagtggctgaaaaagcaaattcaggactggctgcactcattaccgacgggcctggcggaagcaaatggatgtatgttggaaaacaacacgctggcaaaacgttttatgatttaaccggcaatcgaagtgatacagtgacaatcaatgctgatggatggggagaatttaaagtcaatggagggtctgtatccatatgggttccaaaa

SEQ ID NO: 24 - protein, 484 aa, bacillus sp
GSVPVNGTMMQYFEWYLPDDGTLWTKVANNAQSLANLGITALWLPPAYKGTSSSDVGYGVYDLYDLGEFNQKGTVRTKYGTKTQYIQAIQAAHTAGMQVYADVVFNHKAGADGTELVDAVEVNPSDRNQEISGTYQIQAWTKFDFPGRGNTYSSFKWRWYHFDGTDWDESRKLNRIYKFRGTGKAWDWEVDTENGNYDYLMYADLDMDHPEVVSELKNWGKWYVTTTNIDGFRLDAVKHIKYSFFPDWLSYVRTQTQKPLFAVGEFWSYDISKLHNYITKTNGSMSLFDAPLHNNFYIASKSGGYFDMRTLLNNTLMKDQPTLAVTLVDNHDTEPGQSLQSWVEPWFKPLAYAFILTRQEGYPCVFYGDYYGIPKYNIPALKSKLDPLLIARRDYAYGTQHDYIDSADIIGWTREGVAEKANSGLAALITDGPGGSKWMYVGKQHAGKTFYDLTGNRSDTVTINADGWGEFKVNGGSVSIWVPK

SEQ ID NO: 25 - DNA, 1455 bp, Bacillus sp.
  CDS (1)..(1455)
gctaatactgcacctattaacgaaacaatgatgcaatattttgaatgggatttaccgaacgatggaaccctttggacaaaggtgaaaaatgaagccgcaaatctttcttcgctcggtattacagcgttatggcttcctccagcgtataaaggaacaagtcaaagcgatgtcggatacggcgtgtacgatttatatgaccttggggaatttaatcaaaaaggaacgattcgaacaaaatacggaacaaaaacacaatatattcaagccatccaagctgccaaagccgcagggatgcaagtatatgcagatgttgtctttaatcataaggcgggagctgacggcacagaatttgtcgatgcggttgaggtagacccttctaatcgaaatcaagaaacatctggaacatatcaaattcaagcatggacaaaatttgattttcccggtcgggggaacacatactcgagttttaaatggcgttggtatcattttgacggtaccgattgggatgaaagccgaaaattaaatcggatttacaaattccgcagtacaggaaaagcatgggactgggaagtcgatacagaaaacggaaactatgattatttaatgttcgctgatttagatatggatcaccctgaggttgtgacagaattaaaaaactggggaacgtggtacgtcaatactacaaatatcgatggattccgcttagatgccgtaaaacatattaaatacagctttttccctgactggctaacatatgtacgtaatcaaacaggaaaaaatttatttgccgttggggaattttggagctatgacgtcaataagctgcataattacattacaaaaacaaatggatcgatgtcattatttgatgcacctttgcataacaacttttataccgcttccaaatcgagtggatattttgacatgcgttatttattgaataatacattaatgaaagatcaaccttcactcgctgtgacacttgtcgataaccacgacacgcaaccagggcaatctttacagtcatgggtcgaaccttggtttaaaccacttgcttacgcctttattttaacgagacaagagggatatccttgcgtattttacggtgactattatggaatcccgaaatacaatattccaggattaaaaagcaaaatcgacccgcttttaattgctcgtcgggactatgcctatggaacacaacgtgattacattgaccatcaagacattattggatggacacgcgaaggcattgatacaaaaccaaactctggactggcggctttaattaccgacggccctggcggaagcaaatggatgtatgtcggtaaaaaacatgctggaaaagtattttatgatttaaccggaaaccgaagtgacacagtaacgattaatgcggatggttggggagaatttaaagtaaacggaggctccgtttcgatttgggtggctaaa

SEQ ID NO: 26 - protein, 485 aa, Bacillus sp.
ANTAPINETMMQYFEWDLPNDGTLWTKVKNEAANLSSLGITALWLPPAYKGTSQSDVGYGVYDLYDLGEFNQKGTIRTKYGTKTQYIQAIQAAKAAGMQVYADVVFNHKAGADGTEFVDAVEVDPSNRNQETSGTYQIQAWTKFDFPGRGNTYSSFKWRWYHFDGTDWDESRKLNRIYKFRSTGKAWDWEVDTENGNYDYLMFADLDMDHPEVVTELKNWGTWYVNTTNIDGFRLDAVKHIKYSFFPDWLTYVRNQTGKNLFAVGEFWSYDVNKLHNYITKTNGSMSLFDAPLHNNFYTASKSSGYFDMRYLLNNTLMKDQPSLAVTLVDNHDTQPGQSLQSWVEPWFKPLAYAFILTRQEGYPCVFYGDYYGIPKYNIPGLKSKIDPLLIARRDYAYGTQRDYIDHQDIIGWTREGIDTKPNSGLAALITDGPGGSKWMYVGKKHAGKVFYDLTGNRSDTVTINADGWGEFKVNGGSVSIWVAK